European Patent Application EP 4 538 285 A1, published April 16, 2025. Title: PD-1 VARIANT AND USE THEREOF. Applicant: CHINEO MEDICAL TECHNOLOGY CO., LTD. Application EP. The sequence listing filed with the application follows.

SEQUENCE LISTING (63 sequences)

SEQ ID NO: 1 - protein, 288 aa, Homo sapiens
MQIPQAPWPVVWAVLQLGWRPGWFLDSPDRPWNPPTFSPALLVVTEGDNATFTCSFSNTSESFVLNWYRMSPSNQTDKLAAFPEDRSQPGQDCRFRVTQLPNGRDFHMSVVRARRNDSGTYLCGAISLAPKAQIKESLRAELRVTERRAEVPTAHPSPSPRPAGQFQTLVVGVVGGLLGSLVLLVWVLAVICSRAARGTIGARRTGQPLKEDPSAVPVFSVDYGELDFQWREKTPEPPVPCVPEQTEYATIVFPSGMGTSSPARRGSADGPRSAQPLRPEDGHCSWPL

SEQ ID NO: 2 - protein, 155 aa, synthetic construct
  REGION 1..155: note = PD1_56#
MQIPQAPWPVVWAVLQLGWRPGWFLDSPDRPWNPPTFSPALLVVTEGDNATFTCSFSNTSESFVLNWYRMSPSNQTDKLAAFPEDRSQPGQDCRFRVTQLPNGRDFHMSVVRARRNDSGTYLCGAISLSTPVWIKESLRAELRVTERRAEVPTAH

SEQ ID NO: 3 - protein, 155 aa, synthetic construct
  REGION 1..155: note = PD1_56#-2
MQIPQAPWPVVWAVLQLGWRPGWFLDSPDRPWNPPTFSPALLVVTEGDNATFTCSFSNTSESFVLNWYRMSPSNQTDKLAAFPFLFNLPGQDCRFRVTQLPNGRDFHMSVVRARRNDSGTYLCGAISLSTPVWIKESLRAELRVTERRAEVPTAH

SEQ ID NO: 4 - protein, 155 aa, synthetic construct
  REGION 1..155: note = PD1_56#-3
MQIPQAPWPVVWAVLQLGWRPGWFLDSPDRPWNPPTFSPALLVVTEGDNATFTCSFSNTSESFVLNWYRMSPSNQTDKLAAFPWMFCFPGQDCRFRVTQLPNGRDFHMSVVRARRNDSGTYLCGAISLSTPVWIKESLRAELRVTERRAEVPTAH

SEQ ID NO: 5 - protein, 155 aa, synthetic construct
  REGION 1..155: note = PD1_56#-15
MQIPQAPWPVVWAVLQLGWRPGWFLDSPDRPWNPPTFSPALLVVTEGDNATFTCSFSNTSESFVLNWYRMSPSNQTDKLAAFPEDFRNCTQDCRFRVTQLPNGRDFHMSVVRARRNDSGTYLCGAISLSTPVWIKESLRAELRVTERRAEVPTAH

SEQ ID NO: 6 - protein, 155 aa, synthetic construct
  REGION 1..155: note = PD1_56#-16
MQIPQAPWPVVWAVLQLGWRPGWFLDSPDRPWNPPTFSPALLVVTEGDNATFTCSFSNTSESFVLNWYRMSPSNQTDKLAAFPEDFFTVSQDCRFRVTQLPNGRDFHMSVVRARRNDSGTYLCGAISLSTPVWIKESLRAELRVTERRAEVPTAH

SEQ ID NO: 7 - protein, 155 aa, synthetic construct
  REGION 1..155: note = PD1_56#-108
MQIPQAPWPVVWAVLQLGWRPGWFLDSPDRPWNPPTFSPALLVVTEGDNATFTCSFSNTSESFVLNWYRMSPSNQTDKLAAFPEDRINRSQDCRFRVTQLPNGRDFHMSVVRARRNDSGTYLCGAISLSTPVWIKESLRAELRVTERRAEVPTAH

SEQ ID NO: 8 - protein, 155 aa, synthetic construct
  REGION 1..155: note = 56#-2AA
MQIPQAPWPVVWAVLQLGWRPGWFLDSPDRPWNPPTFSPALLVVTEGDNATFTCSFSNTSESFVLNWYRMSPSNQTDKLAAFPFLFNLPGQDCRFRVTQLPNGRDFHMSVVRARRNDSGTYLCGAISLATPAWIKESLRAELRVTERRAEVPTAH

SEQ ID NO: 9 - protein, 155 aa, synthetic construct
  REGION 1..155: note = 56#-15-38
MQIPQAPWPVVWAVLQLGWRPGWFLDSPDRPWNPPTFSPALLVVTEGDNATFTCSFSNTSESFVLNWYRMSPSNQTDKLAAFPEDFRNCTQDCRFRVTQLPNGRDFHMSVVRARRNDSGTYLCGAISLGTPAWIKESLRAELRVTERRAEVPTAH

SEQ ID NO: 10 - protein, 155 aa, synthetic construct
  REGION 1..155: note = 56#-15-61
MQIPQAPWPVVWAVLQLGWRPGWFLDSPDRPWNPPTFSPALLVVTEGDNATFTCSFSNTSESFVLNWYRMSPSNQTDKLAAFPEDFRNCTQDCRFRVTQLPNGRDFHMSVVRARRNDSGTYLCGAISLATPGWIKESLRAELRVTERRAEVPTAH

SEQ ID NO: 11 - protein, 155 aa, synthetic construct
  REGION 1..155: note = 56#-15-69
MQIPQAPWPVVWAVLQLGWRPGWFLDSPDRPWNPPTFSPALLVVTEGDNATFTCSFSNTSESFVLNWYRMSPSNQTDKLAAFPEDFRNCTQDCRFRVTQLPNGRDFHMSVVRARRNDSGTYLCGAISLQTPAWIKESLRAELRVTERRAEVPTAH

SEQ ID NO: 12 - protein, 155 aa, synthetic construct
  REGION 1..155: note = 56#-15-68
MQIPQAPWPVVWAVLQLGWRPGWFLDSPDRPWNPPTFSPALLVVTEGDNATFTCSFSNTSESFVLNWYRMSPSNQTDKLAAFPEDFFTVSQDCRFRVTQLPNGRDFHMSVVRARRNDSGTYLCGAISLYTPAWIKESLRAELRVTERRAEVPTAH

SEQ ID NO: 13 - protein, 155 aa, synthetic construct
  REGION 1..155: note = PD1_49#
MQIPQAPWPVVWAVLQLGWRPGWFLDSPDRPWNPPTFSPALLVVTEGDNATFTCSFSNTSESFVLNWYRMSPSNQTDKLAAFPEDRSQPGQDCRFRVTQLPNGRDFHMSVVRARRNDSGTYLCGAISLHFRFNIKESLRAELRVTERRAEVPTAH

SEQ ID NO: 14 - protein, 155 aa, synthetic construct
  REGION 1..155: note = PD1_110#
MQIPQAPWPVVWAVLQLGWRPGWFLDSPDRPWNPPTFSPALLVVTEGDNATFTCSFSNTSESFVLNWYRMSPSNQTDKLAAFPEDRSQPGQDCRFRVTQLPNGRDFHMSVVRARRNDSGTYLCGAISLSEPIVIKESLRAELRVTERRAEVPTAH

SEQ ID NO: 15 - protein, 155 aa, synthetic construct
  REGION 1..155: note = PD1_49#_93
MQIPQAPWPVVWAVLQLGWRPGWFLDSPDRPWNPPTFSPALLVVTEGDNATFTCSFSNTSESFVLNWYRMSPSNQTDKLAAFPEDRLCVFQDCRFRVTQLPNGRDFHMSVVRARRNDSGTYLCGAISLHFRFNIKESLRAELRVTERRAEVPTAH

SEQ ID NO: 16 - protein, 155 aa, synthetic construct
  REGION 1..155: note = PD1_49#_260
MQIPQAPWPVVWAVLQLGWRPGWFLDSPDRPWNPPTFSPALLVVTEGDNATFTCSFSNTSESFVLNWYRMSPSNQTDKLAAFPEDSFEVRQDCRFRVTQLPNGRDFHMSVVRARRNDSGTYLCGAISLHFRFNIKESLRAELRVTERRAEVPTAH

SEQ ID NO: 17 - protein, 155 aa, synthetic construct
  REGION 1..155: note = PD1_110#_48
MQIPQAPWPVVWAVLQLGWRPGWFLDSPDRPWNPPTFSPALLVVTEGDNATFTCSFSNTSESFVLNWYRMSPSNQTDKLAAFPEDLYLKYQDCRFRVTQLPNGRDFHMSVVRARRNDSGTYLCGAISLSEPIVIKESLRAELRVTERRAEVPTAH

SEQ ID NO: 18 - protein, 155 aa, synthetic construct
  REGION 1..155: note = 56#-15-7
MQIPQAPWPVVWAVLQLGWRPGWFLDSPDRPWNPPTFSPALLVVTEGDNATFTCSFSNTSESFVLNWYRMSPSNQTDKLAAFPEDFRNCTQDCRFRVTQLPNGRDFHMSVVRARRNDSGTYLCGAISLWTPMWIKESLRAELRVTERRAEVPTAH

SEQ ID NO: 19 - protein, 155 aa, synthetic construct
  REGION 1..155: note = 56#-16-12
MQIPQAPWPVVWAVLQLGWRPGWFLDSPDRPWNPPTFSPALLVVTEGDNATFTCSFSNTSESFVLNWYRMSPSNQTDKLAAFPEDFFTVSQDCRFRVTQLPNGRDFHMSVVRARRNDSGTYLCGAISLHTPFWIKESLRAELRVTERRAEVPTAH

SEQ ID NO: 20 - protein, 155 aa, synthetic construct
  REGION 1..155: note = 56#-16-13
MQIPQAPWPVVWAVLQLGWRPGWFLDSPDRPWNPPTFSPALLVVTEGDNATFTCSFSNTSESFVLNWYRMSPSNQTDKLAAFPEDFFTVSQDCRFRVTQLPNGRDFHMSVVRARRNDSGTYLCGAISLGTPFWIKESLRAELRVTERRAEVPTAH

SEQ ID NO: 21 - protein, 155 aa, synthetic construct
  REGION 1..155: note = 56#-16-50
MQIPQAPWPVVWAVLQLGWRPGWFLDSPDRPWNPPTFSPALLVVTEGDNATFTCSFSNTSESFVLNWYRMSPSNQTDKLAAFPEDFFTVSQDCRFRVTQLPNGRDFHMSVVRARRNDSGTYLCGAISLITPGWIKESLRAELRVTERRAEVPTAH

SEQ ID NO: 22 - protein, 155 aa, synthetic construct
  REGION 1..155: note = 56#-108-51
MQIPQAPWPVVWAVLQLGWRPGWFLDSPDRPWNPPTFSPALLVVTEGDNATFTCSFSNTSESFVLNWYRMSPSNQTDKLAAFPEDRINRSQDCRFRVTQLPNGRDFHMSVVRARRNDSGTYLCGAISLTTPFWIKESLRAELRVTERRAEVPTAH

SEQ ID NO: 23 - protein, 155 aa, synthetic construct
  REGION 1..155: note = 56#-108-60
MQIPQAPWPVVWAVLQLGWRPGWFLDSPDRPWNPPTFSPALLVVTEGDNATFTCSFSNTSESFVLNWYRMSPSNQTDKLAAFPEDRINRSQDCRFRVTQLPNGRDFHMSVVRARRNDSGTYLCGAISLVTPAWIKESLRAELRVTERRAEVPTAH

SEQ ID NO: 24 - protein, 155 aa, synthetic construct
  REGION 1..155: note = 56#-108AA
MQIPQAPWPVVWAVLQLGWRPGWFLDSPDRPWNPPTFSPALLVVTEGDNATFTCSFSNTSESFVLNWYRMSPSNQTDKLAAFPEDRINRSQDCRFRVTQLPNGRDFHMSVVRARRNDSGTYLCGAISLATPAWIKESLRAELRVTERRAEVPTAH

SEQ ID NO: 25 - protein, 155 aa, synthetic construct
  REGION 1..155: note = 56#-15AA
MQIPQAPWPVVWAVLQLGWRPGWFLDSPDRPWNPPTFSPALLVVTEGDNATFTCSFSNTSESFVLNWYRMSPSNQTDKLAAFPEDFRNCTQDCRFRVTQLPNGRDFHMSVVRARRNDSGTYLCGAISLATPAWIKESLRAELRVTERRAEVPTAH

SEQ ID NO: 26 - protein, 155 aa, synthetic construct
  REGION 1..155: note = 56#-16AA
MQIPQAPWPVVWAVLQLGWRPGWFLDSPDRPWNPPTFSPALLVVTEGDNATFTCSFSNTSESFVLNWYRMSPSNQTDKLAAFPEDFFTVSQDCRFRVTQLPNGRDFHMSVVRARRNDSGTYLCGAISLATPAWIKESLRAELRVTERRAEVPTAH

SEQ ID NO: 27 - DNA, 57 bp, synthetic construct
  misc_feature 1..57: note = 7074-For
  misc_feature 19..20: note = n is a, c, g, or t
  misc_feature 22..23: note = n is a, c, g, or t
  misc_feature 25..26: note = n is a, c, g, or t
  misc_feature 28..29: note = n is a, c, g, or t
  misc_feature 31..32: note = n is a, c, g, or t
  source 1..57: mol_type = other DNA
gtgctaaactggtaccgcnnknnknnknnknnkcagacggacaagctggccgccttc

SEQ ID NO: 28 - DNA, 22 bp, synthetic construct
  misc_feature 1..22: note = 7074-Rev
  source 1..22: mol_type = other DNA
gcggtaccagtttagcacgaag

SEQ ID NO: 29 - DNA, 51 bp, synthetic construct
  misc_feature 1..51: note = 7478-For
  misc_feature 19..20: note = n is a, c, g, or t
  misc_feature 22..23: note = n is a, c, g, or t
  misc_feature 25..26: note = n is a, c, g, or t
  misc_feature 28..29: note = n is a, c, g, or t
  misc_feature 31..32: note = n is a, c, g, or t
  source 1..51: mol_type = other DNA
taccgcatgagccccagcnnknnknnknnknnkctggccgccttccccgag

SEQ ID NO: 30 - DNA, 19 bp, synthetic construct
  misc_feature 1..19: note = 7478-Rev
  source 1..19: mol_type = other DNA
gctggggctcatgcggtac

SEQ ID NO: 31 - DNA, 54 bp, synthetic construct
  misc_feature 1..54: note = 12731-For
  misc_feature 19..20: note = n is a, c, g, or t
  misc_feature 22..23: note = n is a, c, g, or t
  misc_feature 25..26: note = n is a, c, g, or t
  misc_feature 28..29: note = n is a, c, g, or t
  misc_feature 31..32: note = n is a, c, g, or t
  source 1..54: mol_type = other DNA
tacctctgtggggccatcnnknnknnknnknnkgcgcagatcaaagagagcctg

SEQ ID NO: 32 - DNA, 22 bp, synthetic construct
  misc_feature 1..22: note = 12731-Rev
  source 1..22: mol_type = other DNA
gatggccccacagaggtaggtg

SEQ ID NO: 33 - DNA, 55 bp, synthetic construct
  misc_feature 1..55: note = 12933-For
  misc_feature 19..20: note = n is a, c, g, or t
  misc_feature 22..23: note = n is a, c, g, or t
  misc_feature 25..26: note = n is a, c, g, or t
  misc_feature 28..29: note = n is a, c, g, or t
  misc_feature 31..32: note = n is a, c, g, or t
  source 1..55: mol_type = other DNA
tgtggggccatctccctgnnknnknnknnknnkatcaaagagagcctgcgggcag

SEQ ID NO: 34 - DNA, 21 bp, synthetic construct
  misc_feature 1..21: note = 12933-Rev
  source 1..21: mol_type = other DNA
cagggagatggccccacagag

SEQ ID NO: 35 - DNA, 30 bp, synthetic construct
  misc_feature 1..30: note = P1-For
  source 1..30: mol_type = other DNA
tagctctagaccaccatgcagatcccacag

SEQ ID NO: 36 - DNA, 27 bp, synthetic construct
  misc_feature 1..27: note = P1-Rev
  source 1..27: mol_type = other DNA
gattgtcgacttaggagcgataggctg

SEQ ID NO: 37 - DNA, 55 bp, synthetic construct
  misc_feature 1..55: note = 8488-For
  misc_feature 20..21: note = n is a, c, g, or t
  misc_feature 23..24: note = n is a, c, g, or t
  misc_feature 26..27: note = n is a, c, g, or t
  misc_feature 29..30: note = n is a, c, g, or t
  misc_feature 32..33: note = n is a, c, g, or t
  source 1..55: mol_type = other DNA
caagctggccgccttccccnnknnknnknnknnkcccggccaggactgccgcttc

SEQ ID NO: 38 - DNA, 21 bp, synthetic construct
  misc_feature 1..21: note = 8488-Rev
  source 1..21: mol_type = other DNA
ggggaaggcggccagcttgtc

SEQ ID NO: 39 - DNA, 56 bp, synthetic construct
  misc_feature 1..56: note = 8690-For
  misc_feature 21..22: note = n is a, c, g, or t
  misc_feature 24..25: note = n is a, c, g, or t
  misc_feature 27..28: note = n is a, c, g, or t
  misc_feature 30..31: note = n is a, c, g, or t
  misc_feature 33..34: note = n is a, c, g, or t
  source 1..56: mol_type = other DNA
tggccgccttccccgaggacnnknnknnknnknnkcaggactgccgcttccgtgtc

SEQ ID NO: 40 - DNA, 21 bp, synthetic construct
  misc_feature 1..21: note = 8690-Rev
  source 1..21: mol_type = other DNA
gtcctcggggaaggcggccag

SEQ ID NO: 41 - DNA, 1812 bp, synthetic construct
  misc_feature 1..1812: note = ESO1-TCR
  source 1..1812: mol_type = other DNA
atggagaccctcttgggcctgcttatcctttggctgcagctgcaatgggtgagcagcaaacaggaggtgacgcagattcctgcagctctgagtgtcccagaaggagaaaacttggttctcaactgcagtttcactgatagcgctatttacaacctccagtggtttaggcaggaccctgggaaaggtctcacatctctgttgcttattcagtcaagtcagagagagcaaacaagtggaagacttaatgcctcgctggataaatcatcaggacgtagtactttatacattgcagcttctcagcctggtgactcagccacctacctctgtgctgtgaggcccttatacggaggaagctacatacctacatttggaagaggaaccagccttattgttcatccgtacatccagaaccctgaccctgccgtgtaccagctgagagactctaaatccagtgacaagtctgtctgcctattcaccgattttgattctcaaacaaatgtgtcacaaagtaaggattctgatgtgtatatcacagacaaaactgtgctagacatgaggtctatggacttcaagagcaacagtgctgtggcctggagcaacaaatctgactttgcatgtgcaaacgccttcaacaacagcattattccagaagacaccttcttccccagcccagaaagttcctgtgatgtcaagctggtcgagaaaagctttgaaacagatacgaacctaaactttcaaaacctgtcagtgattgggttccgaatcctcctcctgaaagtggccgggtttaatctgctcatgacgctgcggctgtggtccagccaatgtactaactacgctttgttgaaactcgctggcgatgttgaaagtaaccccggtcctatgagcatcggcctcctgtgctgtgcagccttgtctctcctgtgggcaggtccagtgaatgctggtgtcactcagaccccaaaattccaggtcctgaagacaggacagagcatgacactgcagtgtgcccaggatatgaaccatgaatacatgtcctggtatcgacaagacccaggcatggggctgaggctgattcattactcagttggtgctggtatcactgaccaaggagaagtccccaatggctacaatgtctccagatcaaccacagaggatttcccgctcaggctgctgtcggctgctccctcccagacatctgtgtacttctgtgccagcagttacgtcgggaacaccggggagctgttttttggagaaggctctaggctgaccgtactggaggacctgaagaacgtgttcccacccgaggtcgctgtgtttgagccatcagaagcagagatctcccacacccaaaaggccacactggtgtgcctggccacaggcttcttccctgaccacgtggagctgagctggtgggtgaatgggaaggaggtgcacagtggggtcagcacggacccgcagcccctcaaggagcagcccgccctcaatgactccagatactgcctgagcagccgcctgagggtctcggccaccttctggcagaacccccgcaaccacttccgctgtcaagtccagttctacgggctctcggagaatgacgagtggacccaggatagggccaaacccgtcacccagatcgtcagcgccgaggcctggggtagagcagactgtggctttacctcggtgtcctaccagcaaggggtcctgtctgccaccatcctctatgagatcctgctagggaaggccaccctgtatgctgtgctggtcagcgcccttgtgttgatggccatggtcaagagaaaggatttctaa

SEQ ID NO: 42 - DNA, 2559 bp, synthetic construct
  misc_feature 1..2559: note = 108-CD28-TCR
  source 1..2559: mol_type = other DNA
atgcagatcccacaggcgccctggccagtcgtctgggcggtgctacaactgggctggcggccaggatggttcttagactccccagacaggccctggaacccccccaccttctccccagccctgctcgtggtgaccgaaggggacaacgccaccttcacctgcagcttctccaacacatcggagagcttcgtgctaaactggtaccgcatgagccccagcaaccagacggacaagctggccgccttccccgaggaccgtattaataggagtcaggactgccgcttccgtgtcacacaactgcccaacgggcgtgacttccacatgagcgtggtcagggcccggcgcaatgacagcggcacctacctctgtggggccatctccctgtctactccggtgtggatcaaagagagcctgcgggcagagctcagggtgacagagagaagggcagaagtgcccacagcccaccccagcccctcacccaggccagccggccagttccaaaccctggtggttggtgtcgtgggcggcctgctgggcagcctggtgctgctagtctgggtcctggccgtcatcaggagtaagaggagcaggctcctgcacagtgactacatgaacatgactccccgccgccccgggcccacccgcaagcattaccagccctatgccccaccacgcgacttcgcagcctatcgctccgagggcagaggaagtcttctaacatgcggtgacgtggaggagaatcccggccctatggagaccctcttgggcctgcttatcctttggctgcagctgcaatgggtgagcagcaaacaggaggtgacgcagattcctgcagctctgagtgtcccagaaggagaaaacttggttctcaactgcagtttcactgatagcgctatttacaacctccagtggtttaggcaggaccctgggaaaggtctcacatctctgttgcttattcagtcaagtcagagagagcaaacaagtggaagacttaatgcctcgctggataaatcatcaggacgtagtactttatacattgcagcttctcagcctggtgactcagccacctacctctgtgctgtgaggcccttatacggaggaagctacatacctacatttggaagaggaaccagccttattgttcatccgtacatccagaaccctgaccctgccgtgtaccagctgagagactctaaatccagtgacaagtctgtctgcctattcaccgattttgattctcaaacaaatgtgtcacaaagtaaggattctgatgtgtatatcacagacaaaactgtgctagacatgaggtctatggacttcaagagcaacagtgctgtggcctggagcaacaaatctgactttgcatgtgcaaacgccttcaacaacagcattattccagaagacaccttcttccccagcccagaaagttcctgtgatgtcaagctggtcgagaaaagctttgaaacagatacgaacctaaactttcaaaacctgtcagtgattgggttccgaatcctcctcctgaaagtggccgggtttaatctgctcatgacgctgcggctgtggtccagccaatgtactaactacgctttgttgaaactcgctggcgatgttgaaagtaaccccggtcctatgagcatcggcctcctgtgctgtgcagccttgtctctcctgtgggcaggtccagtgaatgctggtgtcactcagaccccaaaattccaggtcctgaagacaggacagagcatgacactgcagtgtgcccaggatatgaaccatgaatacatgtcctggtatcgacaagacccaggcatggggctgaggctgattcattactcagttggtgctggtatcactgaccaaggagaagtccccaatggctacaatgtctccagatcaaccacagaggatttcccgctcaggctgctgtcggctgctccctcccagacatctgtgtacttctgtgccagcagttacgtcgggaacaccggggagctgttttttggagaaggctctaggctgaccgtactggaggacctgaagaacgtgttcccacccgaggtcgctgtgtttgagccatcagaagcagagatctcccacacccaaaaggccacactggtgtgcctggccacaggcttcttccctgaccacgtggagctgagctggtgggtgaatgggaaggaggtgcacagtggggtcagcacggacccgcagcccctcaaggagcagcccgccctcaatgactccagatactgcctgagcagccgcctgagggtctcggccaccttctggcagaacccccgcaaccacttccgctgtcaagtccagttctacgggctctcggagaatgacgagtggacccaggatagggccaaacccgtcacccagatcgtcagcgccgaggcctggggtagagcagactgtggctttacctcggtgtcctaccagcaaggggtcctgtctgccaccatcctctatgagatcctgctagggaaggccaccctgtatgctgtgctggtcagcgcccttgtgttgatggccatggtcaagagaaaggatttc

SEQ ID NO: 43 - DNA, 43 bp, synthetic construct
  misc_feature 1..43: note = P32-For
  source 1..43: mol_type = other DNA
tcagtagctagcggtaccgccgccaccatgcagatcccacagg

SEQ ID NO: 44 - DNA, 31 bp, synthetic construct
  misc_feature 1..31: note = P32-Rev
  source 1..31: mol_type = other DNA
gttgaggatccgtgggctgtgggcacttctg

SEQ ID NO: 45 - DNA, 1986 bp, synthetic construct
  misc_feature 1..1986: note = PD1-CD3-Fc
  source 1..1986: mol_type = other DNA
aagcttgccgccaccatgcagatcccacaggcgccctggccagtcgtctgggcggtgctacaactgggctggcggccaggatggttcttagactccccagacaggccctggaacccccccaccttctccccagccctgctcgtggtgaccgaaggggacaacgccaccttcacctgcagcttctccaacacatcggagagcttcgtgctaaactggtaccgcatgagccccagcaaccagacggacaagctggccgccttccccgaggaccgtattaataggagtcaggactgccgcttccgtgtcacacaactgcccaacgggcgtgacttccacatgagcgtggtcagggcccggcgcaatgacagcggcacctacctctgtggggccatctccctgtctactccggtgtggatcaaagagagcctgcgggcagagctcagggtgacagagagaagggcagaagtgcccacagcccacggtggcggtggctcgggcggtggtgggtcgggtggcggcggatctgacatccagatgacccagtccccgagctccctgtccgctagcgtgggcgatagggtcaccatcacctgtcgtgccagtcaggacatccgtaattatctcaactggtatcaacagaaaccaggaaaagctccgaaactactgatttactatacctcccgcctggagtctggagtcccttctcgcttctctggttctggttctgggacggattacactctgaccatcagcagtctgcaaccggaggacttcgcaacttattactgtcagcaaggtaatactctgccgtggacgttcggacagggcaccaaggtggagatcaaaggtggaggcggttcaggcggaggtggctctggcggtggcggatcggaggttcagctggtggagtctggcggtggcctggtgcagccagggggctcactccgtttgtcctgtgcagcttctggctactcctttaccggctacactatgaactgggtgcgtcaggccccaggtaagggcctggaatgggttgcactgattaatccttataaaggtgtttccacctataaccagaaattcaaggatcgtttcacgatatccgtagataaatccaaaaacacagcctacctgcaaatgaacagcctgcgtgctgaggacactgccgtctattattgtgctagaagcggatactacggcgatagcgactggtattttgacgtctggggtcaaggaaccctggtcaccgtctcctcgggcggaggcggaagcggaggaggcggctccggcggaggcgagagcaagtacggccccccttgtcctagctgtcccgctcccgagttcctgggcggccctagcgtgttcctgttccctcccaagcccaaggacaccctgatgatcagcagaacccccgaggtgacctgcgtggtcgtggacgtgagccaagaggaccccgaggtgcagttcaactggtacgtggacggcgtggaggtgcacaacgccaagaccaagcctagagaggagcagttcaacagcacctacagagtggtgagcgtgctgaccgtgctgcaccaagactggctgaacggcaaggagtacaagtgcaaggtgagcaacaagggcctgcctagcagcatcgagaagaccatcagcaaggccaaggggcagcctagagagccccaagtgtacaccctgccccctagccaagaggagatgaccaagaaccaagtgagcctgacctgcctggtgaagggcttctaccctagcgacatcgccgtggagtgggagagcaacgggcagcccgagaacaactacaagaccaccccccccgtgctggacagcgacggcagcttcttcctgtacagcagactgaccgtggacaagagcagatggcaagagggcaacgtgttcagctgcagcgtgatgcacgaggccctgcacaaccactacacacagaagagcctgagcctgagcctgggcaagtaa

SEQ ID NO: 46 - DNA, 1626 bp, synthetic construct
  misc_feature 1..1626: note = LucDNA
  source 1..1626: mol_type = other DNA
atggtaaagcgtgagaaaaatgtcatctatggccctgagcctctccatcctttggaggatttgactgccggcgaaatgctgtttcgtgctctccgcaagcactctcatttgcctcaagccttggtcgatgtggtcggcgatgaatctttgagctacaaggagttttttgaggcaaccgtcttgctggctcagtccctccacaattgtggctacaagatgaacgacgtcgttagtatctgtgctgaaaacaatacccgtttcttcattccagtcatcgccgcatggtatatcggtatgatcgtggctccagtcaacgagagctacattcccgacgaactgtgtaaagtcatgggtatctctaagccacagattgtcttcaccactaagaatattctgaacaaagtcctggaagtccaaagccgcaccaactttattaagcgtatcatcatcttggacactgtggagaatattcacggttgcgaatctttgcctaatttcatctctcgctattcagacggcaacatcgcaaactttaaaccactccacttcgaccctgtggaacaagttgcagccattctgtgtagcagcggtactactggactcccaaagggagtcatgcagacccatcaaaacatttgcgtgcgtctgatccatgctctcgatccacgcgtgggcactcagctgattcctggtgtcaccgtcttggtctacttgcctttcttccatgctttcggctttagcattactttgggttactttatggtcggtctccgcgtgattatgttccgccgttttgatcaggaggctttcttgaaagccatccaagattatgaagtccgcagtgtcatcaacgtgcctagcgtgatcctgtttttgtctaagagcccactcgtggacaagtacgacttgtcttcactgcgtgaattgtgttgcggtgccgctccactggctaaggaggtcgctgaagtggccgccaaacgcttgaatcttccagggattcgttgtggcttcggcctcaccgaatctaccagcgctaacattcactctctcggggatgagtttaagagcggctctttgggccgtgtcactccactcatggctgctaagatcgctgatcgcgaaactggtaaggctttgggcccgaaccaagtgggcgagctgtgtatcaaaggccctatggtgagcaagggttatgtcaataacgttgaagctaccaaggaggccatcgacgacgacggctggttgcattctggtgattttggatattacgacgaagatgagcatttttacgtcgtggatcgttacaaggagctgatcaaatacaagggtagccaggttgctccagctgagttggaggagattctgttgaaaaatccatgcattcgcgatgtcgctgtggtcggcattcctgatctggaggccggcgaactgccttctgctttcgttgtcaagcagcctggtaaagaaattaccgccaaagaagtgtatgattacctggctgaacgtgtgagccatactaagtacttgcgtggcggcgtgcgttttgttgactccatccctcgtaacgtaacaggcaaaattacccgcaaggagctgttgaaacaattgttggagaaggccggcggt

SEQ ID NO: 47 - DNA, 870 bp, synthetic construct
  misc_feature 1..870: note = PD-L1DNA
  source 1..870: mol_type = other DNA
atgaggatatttgctgtctttatattcatgacctactggcatttgctgaacgcatttactgtcacggttcccaaggacctatatgtggtagagtatggtagcaatatgacaattgaatgcaaattcccagtagaaaaacaattagacctggctgcactaattgtctattgggaaatggaggataagaacattattcaatttgtgcatggagaggaagacctgaaggttcagcatagtagctacagacagagggcccggctgttgaaggaccagctctccctgggaaatgctgcacttcagatcacagatgtgaaattgcaggatgcaggggtgtaccgctgcatgatcagctatggtggtgccgactacaagcgaattactgtgaaagtcaatgccccatacaacaaaatcaaccaaagaattttggttgtggatccagtcacctctgaacatgaactgacatgtcaggctgagggctaccccaaggccgaagtcatctggacaagcagtgaccatcaagtcctgagtggtaagaccaccaccaccaattccaagagagaggagaagcttttcaatgtgaccagcacactgagaatcaacacaacaactaatgagattttctactgcacttttaggagattagatcctgaggaaaaccatacagctgaattggtcatcccagaactacctctggcacatcctccaaatgaaaggactcacttggtaattctgggagccatcttattatgccttggtgtagcactgacattcatcttccgtttaagaaaagggagaatgatggatgtgaaaaaatgtggcatccaagatacaaactcaaagaagcaaagtgatacacatttggaggagacg

SEQ ID NO: 48 - protein, 220 aa, synthetic construct
  REGION 1..220: note = PD-L1AA19-238
FTVTVPKDLYVVEYGSNMTIECKFPVEKQLDLAALIVYWEMEDKNIIQFVHGEEDLKVQHSSYRQRARLLKDQLSLGNAALQITDVKLQDAGVYRCMISYGGADYKRITVKVNAPYNKINQRILVVDPVTSEHELTCQAEGYPKAEVIWTSSDHQVLSGKTTTTNSKREEKLFNVTSTLRINTTTNEIFYCTFRRLDPEENHTAELVIPELPLAHPPNER

SEQ ID NO: 49 - protein, 80 aa, synthetic construct
  REGION 1..80: note = CD28TM-ICD
CPSPLFPGPSKPFWVLVVVGGVLACYSLLVTVAFIIFWVRSKRSRLLHSDYMNMTPRRPGPTRKHYQPYAPPRDFAAYRS

SEQ ID NO: 50 - protein, 75 aa, synthetic construct
  REGION 1..75: note = 4-1BBICD
PGHSPQIISFFLALTSTALLFLLFFLTLRFSVVKRGRKKLLYIFKQPFMRPVQTTQEEDGCSCRFPEEEEGGCEL

SEQ ID NO: 51 - protein, 65 aa, synthetic construct
  REGION 1..65: note = OX40ICD
RAVAAILGLGLVLGLLGPLAILLALYLLRRDQRLPPDAHKPPGGGSFRTPIQEEQADAHSTLAKI

SEQ ID NO: 52 - protein, 35 aa, synthetic construct
  REGION 1..35: note = ICOSICD
TKKKYSSSVHDPNGEYMFMRAVNTAKKSRLTDVTL

SEQ ID NO: 53 - protein, 49 aa, synthetic construct
  REGION 1..49: note = CD27ICD
HQRRKYRSNKGESPVEPAEPCHYSCPREEEGSTIPIQEDYRKPEPACSP

SEQ ID NO: 54 - protein, 230 aa, synthetic construct
  REGION 1..230: note = RFc
GSAPSTCSKPTCPPPELLGGPSVFIFPPKPKDTLMISRTPEVTCVVVDVSQDDPEVQFTWYINNEQVRTARPPLREQQFNSTIRVVSTLPIAHQDWLRGKEFKCKVHNKALPAPIEKTISKARGQPLEPKVYTMGPPREELSSRSVSLTCMINGFYPSDISVEWEKNGKAEDNYKTTPAVLDSDGSYFLYSKLSVPTSEWQRGDVFTCSVMHEALHNHYTQKSISRSPGK

SEQ ID NO: 55 - DNA, 465 bp, synthetic construct
  misc_feature 1..465: note = PD1_WTDNA
  source 1..465: mol_type = other DNA
atgcagatcccacaggcgccctggccagtcgtctgggcggtgctacaactgggctggcggccaggatggttcttagactccccagacaggccctggaacccccccaccttctccccagccctgctcgtggtgaccgaaggggacaacgccaccttcacctgcagcttctccaacacatcggagagcttcgtgctaaactggtaccgcatgagccccagcaaccagacggacaagctggccgccttccccgaggaccgcagccagcccggccaggactgccgcttccgtgtcacacaactgcccaacgggcgtgacttccacatgagcgtggtcagggcccggcgcaatgacagcggcacctacctctgtggggccatctccctggcccccaaggcgcagatcaaagagagcctgcgggcagagctcagggtgacagagagaagggcagaagtgcccacagcccac

SEQ ID NO: 56 - DNA, 465 bp, synthetic construct
  misc_feature 1..465: note = PD1_56#
  source 1..465: mol_type = other DNA
atgcagatcccacaggcgccctggccagtcgtctgggcggtgctacaactgggctggcggccaggatggttcttagactccccagacaggccctggaacccccccaccttctccccagccctgctcgtggtgaccgaaggggacaacgccaccttcacctgcagcttctccaacacatcggagagcttcgtgctaaactggtaccgcatgagccccagcaaccagacggacaagctggccgccttccccgaggaccgcagccagcccggccaggactgccgcttccgtgtcacacaactgcccaacgggcgtgacttccacatgagcgtggtcagggcccggcgcaatgacagcggcacctacctctgtggggccatctccctgtctactccggtgtggatcaaagagagcctgcgggcagagctcagggtgacagagagaagggcagaagtgcccacagcccac

SEQ ID NO: 57 - DNA, 465 bp, synthetic construct
  misc_feature 1..465: note = PD1_56#-2
  source 1..465: mol_type = other DNA
atgcagatcccacaggcgccctggccagtcgtctgggcggtgctacaactgggctggcggccaggatggttcttagactccccagacaggccctggaacccccccaccttctccccagccctgctcgtggtgaccgaaggggacaacgccaccttcacctgcagcttctccaacacatcggagagcttcgtgctaaactggtaccgcatgagccccagcaaccagacggacaagctggccgccttcccctttttgtttaatcttcccggccaggactgccgcttccgtgtcacacaactgcccaacgggcgtgacttccacatgagcgtggtcagggcccggcgcaatgacagcggcacctacctctgtggggccatctccctgtctactccggtgtggatcaaagagagcctgcgggcagagctcagggtgacagagagaagggcagaagtgcccacagcccac

SEQ ID NO: 58 - DNA, 465 bp, synthetic construct
  misc_feature 1..465: note = PD1_56#-3
  source 1..465: mol_type = other DNA
atgcagatcccacaggcgccctggccagtcgtctgggcggtgctacaactgggctggcggccaggatggttcttagactccccagacaggccctggaacccccccaccttctccccagccctgctcgtggtgaccgaaggggacaacgccaccttcacctgcagcttctccaacacatcggagagcttcgtgctaaactggtaccgcatgagccccagcaaccagacggacaagctggccgccttcccctggatgttttgttttcccggccaggactgccgcttccgtgtcacacaactgcccaacgggcgtgacttccacatgagcgtggtcagggcccggcgcaatgacagcggcacctacctctgtggggccatctccctgtctactccggtgtggatcaaagagagcctgcgggcagagctcagggtgacagagagaagggcagaagtgcccacagcccac

SEQ ID NO: 59 - DNA, 465 bp, synthetic construct
  misc_feature 1..465: note = PD1_56#-15
  source 1..465: mol_type = other DNA
atgcagatcccacaggcgccctggccagtcgtctgggcggtgctacaactgggctggcggccaggatggttcttagactccccagacaggccctggaacccccccaccttctccccagccctgctcgtggtgaccgaaggggacaacgccaccttcacctgcagcttctccaacacatcggagagcttcgtgctaaactggtaccgcatgagccccagcaaccagacggacaagctggccgccttccccgaggactttaggaattgtacgcaggactgccgcttccgtgtcacacaactgcccaacgggcgtgacttccacatgagcgtggtcagggcccggcgcaatgacagcggcacctacctctgtggggccatctccctgtctactccggtgtggatcaaagagagcctgcgggcagagctcagggtgacagagagaagggcagaagtgcccacagcccac

SEQ ID NO: 60 - DNA, 465 bp, synthetic construct
  misc_feature 1..465: note = PD1_56#-16
  source 1..465: mol_type = other DNA
atgcagatcccacaggcgccctggccagtcgtctgggcggtgctacaactgggctggcggccaggatggttcttagactccccagacaggccctggaacccccccaccttctccccagccctgctcgtggtgaccgaaggggacaacgccaccttcacctgcagcttctccaacacatcggagagcttcgtgctaaactggtaccgcatgagccccagcaaccagacggacaagctggccgccttccccgaggacttttttacggttagtcaggactgccgcttccgtgtcacacaactgcccaacgggcgtgacttccacatgagcgtggtcagggcccggcgcaatgacagcggcacctacctctgtggggccatctccctgtctactccggtgtggatcaaagagagcctgcgggcagagctcagggtgacagagagaagggcagaagtgcccacagcccac

SEQ ID NO: 61 - DNA, 465 bp, synthetic construct
  misc_feature 1..465: note = PD1_56#-108
  source 1..465: mol_type = other DNA
atgcagatcccacaggcgccctggccagtcgtctgggcggtgctacaactgggctggcggccaggatggttcttagactccccagacaggccctggaacccccccaccttctccccagccctgctcgtggtgaccgaaggggacaacgccaccttcacctgcagcttctccaacacatcggagagcttcgtgctaaactggtaccgcatgagccccagcaaccagacggacaagctggccgccttccccgaggaccgtattaataggagtcaggactgccgcttccgtgtcacacaactgcccaacgggcgtgacttccacatgagcgtggtcagggcccggcgcaatgacagcggcacctacctctgtggggccatctccctgtctactccggtgtggatcaaagagagcctgcgggcagagctcagggtgacagagagaagggcagaagtgcccacagcccac

SEQ ID NO: 62 - DNA, 1184 bp, synthetic construct
  misc_feature 1..1184: note = EF1
  source 1..1184: mol_type = other DNA
cgtgaggctccggtgcccgtcagtgggcagagcgcacatcgcccacagtccccgagaagttggggggaggggtcggcaattgaaccggtgcctagagaaggtggcgcggggtaaactgggaaagtgatgtcgtgtactggctccgcctttttcccgagggtgggggagaaccgtatataagtgcagtagtcgccgtgaacgttctttttcgcaacgggtttgccgccagaacacaggtaagtgccgtgtgtggttcccgcgggcctggcctctttacgggttatggcccttgcgtgccttgaattacttccacctggctgcagtacgtgattcttgatcccgagcttcgggttggaagtgggtgggagagttcgaggccttgcgcttaaggagccccttcgcctcgtgcttgagttgaggcctggcctgggcgctggggccgccgcgtgcgaatctggtggcaccttcgcgcctgtctcgctgctttcgataagtctctagccatttaaaatttttgatgacctgctgcgacgctttttttctggcaagatagtcttgtaaatgcgggccaagatctgcacactggtatttcggtttttggggccgcgggcggcgacggggcccgtgcgtcccagcgcacatgttcggcgaggcggggcctgcgagcgcggccaccgagaatcggacgggggtagtctcaagctggccggcctgctctggtgcctggcctcgcgccgccgtgtatcgccccgccctgggcggcaaggctggcccggtcggcaccagttgcgtgagcggaaagatggccgcttcccggccctgctgcagggagctcaaaatggaggacgcggcgctcgggagagcgggcgggtgagtcacccacacaaaggaaaagggcctttccgtcctcagccgtcgcttcatgtgactccactgagtaccgggcgccgtccaggcacctcgattagttctcgtgcttttggagtacgtcgtctttaggttggggggaggggttttatgcgatggagtttccccacactgagtgggtggagactgaagttaggccagcttggcacttgatgtaattctccttggaatttgccctttttgagtttggatcttggttcattctcaagcctcagacagtggttcaaagtttttttcttccatttcaggtgtcgtga

SEQ ID NO: 63 - DNA, 8417 bp, synthetic construct
  misc_feature 1..8417: note = pLV2-PD1-CD28
  source 1..8417: mol_type = other DNA
ttttaaaagaaaaggggggattggggggtacagtgcaggggaaagaatagtagacataatagcaacagacatacaaactaaagaattacaaaaacaaattacaaaaattcaaaattttcgggtttattacagggacagcagagatccagtttggctgcatacgcgtcgtgaggctccggtgcccgtcagtgggcagagcgcacatcgcccacagtccccgagaagttggggggaggggtcggcaattgaaccggtgcctagagaaggtggcgcggggtaaactgggaaagtgatgtcgtgtactggctccgcctttttcccgagggtgggggagaaccgtatataagtgcagtagtcgccgtgaacgttctttttcgcaacgggtttgccgccagaacacaggtaagtgccgtgtgtggttcccgcgggcctggcctctttacgggttatggcccttgcgtgccttgaattacttccacctggctgcagtacgtgattcttgatcccgagcttcgggttggaagtgggtgggagagttcgaggccttgcgcttaaggagccccttcgcctcgtgcttgagttgaggcctggcctgggcgctggggccgccgcgtgcgaatctggtggcaccttcgcgcctgtctcgctgctttcgataagtctctagccatttaaaatttttgatgacctgctgcgacgctttttttctggcaagatagtcttgtaaatgcgggccaagatctgcacactggtatttcggtttttggggccgcgggcggcgacggggcccgtgcgtcccagcgcacatgttcggcgaggcggggcctgcgagcgcggccaccgagaatcggacgggggtagtctcaagctggccggcctgctctggtgcctggcctcgcgccgccgtgtatcgccccgccctgggcggcaaggctggcccggtcggcaccagttgcgtgagcggaaagatggccgcttcccggccctgctgcagggagctcaaaatggaggacgcggcgctcgggagagcgggcgggtgagtcacccacacaaaggaaaagggcctttccgtcctcagccgtcgcttcatgtgactccactgagtaccgggcgccgtccaggcacctcgattagttctcgtgcttttggagtacgtcgtctttaggttggggggaggggttttatgcgatggagtttccccacactgagtgggtggagactgaagttaggccagcttggcacttgatgtaattctccttggaatttgccctttttgagtttggatcttggttcattctcaagcctcagacagtggttcaaagtttttttcttccatttcaggtgtcgtgagctagctctagaccaccatgcagatcccacaggcgccctggccagtcgtctgggcggtgctacaactgggctggcggccaggatggttcttagactccccagacaggccctggaacccccccaccttctccccagccctgctcgtggtgaccgaaggggacaacgccaccttcacctgcagcttctccaacacatcggagagcttcgtgctaaactggtaccgcatgagccccagcaaccagacggacaagctggccgccttccccgaggaccgcagccagcccggccaggactgccgcttccgtgtcacacaactgcccaacgggcgtgacttccacatgagcgtggtcagggcccggcgcaatgacagcggcacctacctctgtggggccatctccctggcccccaaggcgcagatcaaagagagcctgcgggcagagctcagggtgacagagagaagggcagaagtgcccacagcccaccccagcccctcacccaggccagccggccagttccaaaccctggtggttggtgtcgtgggcggcctgctgggcagcctggtgctgctagtctgggtcctggccgtcatcaggagtaagaggagcaggctcctgcacagtgactacatgaacatgactccccgccgccccgggcccacccgcaagcattaccagccctatgccccaccacgcgacttcgcagcctatcgctcctaagtcgacaatcaacctctggattacaaaatttgtgaaagattgactggtattcttaactatgttgctccttttacgctatgtggatacgctgctttaatgcctttgtatcatgctattgcttcccgtatggctttcattttctcctccttgtataaatcctggttgctgtctctttatgaggagttgtggcccgttgtcaggcaacgtggcgtggtgtgcactgtgtttgctgacgcaacccccactggttggggcattgccaccacctgtcagctcctttccgggactttcgctttccccctccctattgccacggcggaactcatcgccgcctgccttgcccgctgctggacaggggctcggctgttgggcactgacaattccgtggtgttgtcggggaagctgacgtcctttccatggctgctcgcctgtgttgccacctggattctgcgcgggacgtccttctgctacgtcccttcggccctcaatccagcggaccttccttcccgcggcctgctgccggctctgcggcctcttccgcgtcttcgccttcgccctcagacgagtcggatctccctttgggccgcctccccgcctggaattcgagctcggtacctttaagaccaatgacttacaaggcagctgtagatcttagccactttttaaaagaaaaggggggactggaagggctaattcactcccaacgaagacaagatctgctttttgcttgtactgggtctctctggttagaccagatctgagcctgggagctctctggctaactagggaacccactgcttaagcctcaataaagcttgccttgagtgcttcaagtagtgtgtgcccgtctgttgtgtgactctggtaactagagatccctcagacccttttagtcagtgtggaaaatctctagcagtagtagttcatgtcatcttattattcagtatttataacttgcaaagaaatgaatatcagagagtgagaggaacttgtttattgcagcttataatggttacaaataaagcaatagcatcacaaatttcacaaataaagcatttttttcactgcattctagttgtggtttgtccaaactcatcaatgtatcttatcatgtctggctctagctatcccgcccctaactccgcccatcccgcccctaactccgcccagttccgcccattctccgccccatggctgactaattttttttatttatgcagaggccgaggccgcctcggcctctgagctattccagaagtagtgaggaggcttttttggaggcctagggacgtacccaattcgccctatagtgagtcgtattacgcgcgctcactggccgtcgttttacaacgtcgtgactgggaaaaccctggcgttacccaacttaatcgccttgcagcacatccccctttcgccagctggcgtaatagcgaagaggcccgcaccgatcgcccttcccaacagttgcgcagcctgaatggcgaatgggacgcgccctgtagcggcgcattaagcgcggcgggtgtggtggttacgcgcagcgtgaccgctacacttgccagcgccctagcgcccgctcctttcgctttcttcccttcctttctcgccacgttcgccggctttccccgtcaagctctaaatcgggggctccctttagggttccgatttagtgctttacggcacctcgaccccaaaaaacttgattagggtgatggttcacgtagtgggccatcgccctgatagacggtttttcgccctttgacgttggagtccacgttctttaatagtggactcttgttccaaactggaacaacactcaaccctatctcggtctattcttttgatttataagggattttgccgatttcggcctattggttaaaaaatgagctgatttaacaaaaatttaacgcgaattttaacaaaatattaacgcttacaatttaggtggcacttttcggggaaatgtgcgcggaacccctatttgtttatttttctaaatacattcaaatatgtatccgctcatgagacaataaccctgataaatgcttcaataatattgaaaaaggaagagtatgagtattcaacatttccgtgtcgcccttattcccttttttgcggcattttgccttcctgtttttgctcacccagaaacgctggtgaaagtaaaagatgctgaagatcagttgggtgcacgagtgggttacatcgaactggatctcaacagcggtaagatccttgagagttttcgccccgaagaacgttttccaatgatgagcacttttaaagttctgctatgtggcgcggtattatcccgtattgacgccgggcaagagcaactcggtcgccgcatacactattctcagaatgacttggttgagtactcaccagtcacagaaaagcatcttacggatggcatgacagtaagagaattatgcagtgctgccataaccatgagtgataacactgcggccaacttacttctgacaacgatcggaggaccgaaggagctaaccgcttttttgcacaacatgggggatcatgtaactcgccttgatcgttgggaaccggagctgaatgaagccataccaaacgacgagcgtgacaccacgatgcctgtagcaatggcaacaacgttgcgcaaactattaactggcgaactacttactctagcttcccggcaacaattaatagactggatggaggcggataaagttgcaggaccacttctgcgctcggcccttccggctggctggtttattgctgataaatctggagccggtgagcgtgggtctcgcggtatcattgcagcactggggccagatggtaagccctcccgtatcgtagttatctacacgacggggagtcaggcaactatggatgaacgaaatagacagatcgctgagataggtgcctcactgattaagcattggtaactgtcagaccaagtttactcatatatactttagattgatttaaaacttcatttttaatttaaaaggatctaggtgaagatcctttttgataatctcatgaccaaaatcccttaacgtgagttttcgttccactgagcgtcagaccccgtagaaaagatcaaaggatcttcttgagatcctttttttctgcgcgtaatctgctgcttgcaaacaaaaaaaccaccgctaccagcggtggtttgtttgccggatcaagagctaccaactctttttccgaaggtaactggcttcagcagagcgcagataccaaatactgttcttctagtgtagccgtagttaggccaccacttcaagaactctgtagcaccgcctacatacctcgctctgctaatcctgttaccagtggctgctgccagtggcgataagtcgtgtcttaccgggttggactcaagacgatagttaccggataaggcgcagcggtcgggctgaacggggggttcgtgcacacagcccagcttggagcgaacgacctacaccgaactgagatacctacagcgtgagctatgagaaagcgccacgcttcccgaagggagaaaggcggacaggtatccggtaagcggcagggtcggaacaggagagcgcacgagggagcttccagggggaaacgcctggtatctttatagtcctgtcgggtttcgccacctctgacttgagcgtcgatttttgtgatgctcgtcaggggggcggagcctatggaaaaacgccagcaacgcggcctttttacggttcctggccttttgctggccttttgctcacatgttctttcctgcgttatcccctgattctgtggataaccgtattaccgcctttgagtgagctgataccgctcgccgcagccgaacgaccgagcgcagcgagtcagtgagcgaggaagcggaagagcgcccaatacgcaaaccgcctctccccgcgcgttggccgattcattaatgcagctggcacgacaggtttcccgactggaaagcgggcagtgagcgcaacgcaattaatgtgagttagctcactcattaggcaccccaggctttacactttatgcttccggctcgtatgttgtgtggaattgtgagcggataacaatttcacacaggaaacagctatgaccatgattacgccaagcgcgcaattaaccctcactaaagggaacaaaagctggagctgcaagcttaatgtagtcttatgcaatactcttgtagtcttgcaacatggtaacgatgagttagcaacatgccttacaaggagagaaaaagcaccgtgcatgccgattggtggaagtaaggtggtacgatcgtgccttattaggaaggcaacagacgggtctgacatggattggacgaaccactgaattgccgcattgcagagatattgtatttaagtgcctagctcgatacataaacgggtctctctggttagaccagatctgagcctgggagctctctggctaactagggaacccactgcttaagcctcaataaagcttgccttgagtgcttcaagtagtgtgtgcccgtctgttgtgtgactctggtaactagagatccctcagacccttttagtcagtgtggaaaatctctagcagtggcgcccgaacagggacttgaaagcgaaagggaaaccagaggagctctctcgacgcaggactcggcttgctgaagcgcgcacggcaagaggcgaggggcggcgactggtgagtacgccaaaaattttgactagcggaggctagaaggagagagatgggtgcgagagcgtcagtattaagcgggggagaattagatcgcgatgggaaaaaattcggttaaggccagggggaaagaaaaaatataaattaaaacatatagtatgggcaagcagggagctagaacgattcgcagttaatcctggcctgttagaaacatcagaaggctgtagacaaatactgggacagctacaaccatcccttcagacaggatcagaagaacttagatcattatataatacagtagcaaccctctattgtgtgcatcaaaggatagagataaaagacaccaaggaagctttagacaagatagaggaagagcaaaacaaaagtaagaccaccgcacagcaagcggccgctgatcttcagacctggaggaggagatatgagggacaattggagaagtgaattatataaatataaagtagtaaaaattgaaccattaggagtagcacccaccaaggcaaagagaagagtggtgcagagagaaaaaagagcagtgggaataggagctttgttccttgggttcttgggagcagcaggaagcactatgggcgcagcgtcaatgacgctgacggtacaggccagacaattattgtctggtatagtgcagcagcagaacaatttgctgagggctattgaggcgcaacagcatctgttgcaactcacagtctggggcatcaagcagctccaggcaagaatcctggctgtggaaagatacctaaaggatcaacagctcctggggatttggggttgctctggaaaactcatttgcaccactgctgtgccttggaatgctagttggagtaataaatctctggaacagatttggaatcacacgacctggatggagtgggacagagaaattaacaattacacaagcttaatacactccttaattgaagaatcgcaaaaccagcaagaaaagaatgaacaagaattattggaattagataaatgggcaagtttgtggaattggtttaacataacaaattggctgtggtatataaaattattcataatgatagtaggaggcttggtaggtttaagaatagtttttgctgtactttctatagtgaatagagttaggcagggatattcaccattatcgtttcagacccacctcccaaccccgaggggacccgacaggcccgaaggaatagaagaagaaggtggagagagagacagagacagatccattcgattagtgaacggatctcgacggtatcgattagactgtagcccaggaatatggcagctagattgtacacatttagaaggaaaagttatcttggtagcagttcatgtagccagtggatatatagaagcagaagtaattccagcagagacagggcaagaaacagcatacttcctcttaaaattagcaggaagatggccagtaaaaacagtacatacagacaatggcagcaatttcaccagtactacagttaaggccgcctgttggtgggcggggatcaagcaggaatttggcattccctacaatccccaaagtcaaggagtaatagaatctatgaataaagaattaaagaaaattataggacaggtaagagatcaggctgaacatcttaagacagcagtacaaatggcagtattcatccacaa